European Patent Application EP 4 487 834 A1, published January 8, 2025. Title: CONSENSUS PEPTIDES IN HYA. Applicant: NuPep AS. The sequence listing filed with the application follows.

SEQUENCE LISTING (7 sequences)

SEQ ID NO: 1 - protein, 92 aa, synthetic construct
  VARIANT 2: note = variant selected from the group consisting of Ala, Ile, Leu, Met, Phe, Trp and Val
  VARIANT 3: note = variant selected from the group consisting of Ala, Ile, Leu, Met, Phe, Trp and Val
  VARIANT 9: note = variant selected from the group consisting of Ala, Ile, Leu, Met, Phe, Trp and Val
  VARIANT 10: note = variant selected from the group consisting of Ala, Ile, Leu, Met, Phe, Trp and Val
  VARIANT 15: note = variant selected from the group consisting of Ala, Ile, Leu, Met, Phe, Trp and Val
  VARIANT 16: note = variant selected from the group consisting of Ala, Ile, Leu, Met, Phe, Trp and Val
  VARIANT 18: note = variant selected from the group consisting of Ala, Ile, Leu, Met, Phe, Trp and Val
  VARIANT 34: note = variant selected from the group consisting of Ala, Ile, Leu, Met, Phe, Trp and Val
  VARIANT 35: note = variant selected from the group consisting of Ala, Ile, Leu, Met, Phe, Trp and Val
  VARIANT 37: note = variant selected from the group consisting of Ala, Ile, Leu, Met, Phe, Trp and Val
  VARIANT 48: note = variant selected from the group consisting of Ala, Ile, Leu, Met, Phe, Trp and Val
  VARIANT 49: note = variant selected from the group consisting of Ala, Ile, Leu, Met, Phe, Trp and Val
  VARIANT 56: note = variant selected from the group consisting of Ala, Ile, Leu, Met, Phe, Trp and Val
  VARIANT 57: note = variant selected from the group consisting of Ala, Ile, Leu, Met, Phe, Trp and Val
  VARIANT 62: note = variant selected from the group consisting of Ala, Ile, Leu, Met, Phe, Trp and Val
  VARIANT 63: note = variant selected from the group consisting of Ala, Ile, Leu, Met, Phe, Trp and Val
  VARIANT 68: note = variant selected from the group consisting of Ala, Ile, Leu, Met, Phe, Trp and Val
  VARIANT 69: note = variant selected from the group consisting of Ala, Ile, Leu, Met, Phe, Trp and Val
  VARIANT 74: note = variant selected from the group consisting of Ala, Ile, Leu, Met, Phe, Trp and Val
  VARIANT 77: note = variant selected from the group consisting of Ala, Ile, Leu, Met, Phe, Trp and Val
  VARIANT 78: note = variant selected from the group consisting of Ala, Ile, Leu, Met, Phe, Trp and Val
  VARIANT 79: note = variant selected from the group consisting of Ala, Ile, Leu, Met, Phe, Trp and Val
  VARIANT 80: note = variant selected from the group consisting of Ala, Ile, Leu, Met, Phe, Trp and Val
  VARIANT 81: note = variant selected from the group consisting of Ala, Ile, Leu, Met, Phe, Trp and Val
  VARIANT 82: note = variant selected from the group consisting of Ala, Ile, Leu, Met, Phe, Trp and Val
  VARIANT 83: note = variant selected from the group consisting of Ala, Ile, Leu, Met, Phe, Trp and Val
  VARIANT 84: note = variant selected from the group consisting of Ala, Ile, Leu, Met, Phe, Trp and Val
  VARIANT 89: note = variant selected from the group consisting of Ala, Ile, Leu, Met, Phe, Trp and Val
  VARIANT 90: note = variant selected from the group consisting of Ala, Ile, Leu, Met, Phe, Trp and Val
  VARIANT 91: note = variant selected from the group consisting of Ala, Ile, Leu, Met, Phe, Trp and Val
  VARIANT 92: note = variant selected from the group consisting of Ala, Ile, Leu, Met, Phe, Trp and Val
  VARIANT 86: note = variant selected from the group consisting of Ala, Ile, Leu, Met, Phe, Trp and Val
  VARIANT 87: note = variant selected from the group consisting of Ala, Ile, Leu, Met, Phe, Trp and Val
  VARIANT 5: note = variant selected from the group consisting of Asn, Cys, Gln, Ser, Thr and Tyr
  VARIANT 6: note = variant selected from the group consisting of Asn, Cys, Gln, Ser, Thr and Tyr
  VARIANT 7: note = variant selected from the group consisting of Asn, Cys, Gln, Ser, Thr and Tyr
  VARIANT 12: note = variant selected from the group consisting of Asn, Cys, Gln, Ser, Thr and Tyr
  VARIANT 13: note = variant selected from the group consisting of Asn, Cys, Gln, Ser, Thr and Tyr
  VARIANT 20: note = variant selected from the group consisting of Asn, Cys, Gln, Ser, Thr and Tyr
  VARIANT 21: note = variant selected from the group consisting of Asn, Cys, Gln, Ser, Thr and Tyr
  VARIANT 22: note = variant selected from the group consisting of Asn, Cys, Gln, Ser, Thr and Tyr
  VARIANT 23: note = variant selected from the group consisting of Asn, Cys, Gln, Ser, Thr and Tyr
  VARIANT 24: note = variant selected from the group consisting of Asn, Cys, Gln, Ser, Thr and Tyr
  VARIANT 25: note = variant selected from the group consisting of Asn, Cys, Gln, Ser, Thr and Tyr
  VARIANT 27: note = variant selected from the group consisting of Asn, Cys, Gln, Ser, Thr and Tyr
  VARIANT 28: note = variant selected from the group consisting of Asn, Cys, Gln, Ser, Thr and Tyr
  VARIANT 29: note = variant selected from the group consisting of Asn, Cys, Gln, Ser, Thr and Tyr
  VARIANT 30: note = variant selected from the group consisting of Asn, Cys, Gln, Ser, Thr and Tyr
  VARIANT 32: note = variant selected from the group consisting of Asn, Cys, Gln, Ser, Thr and Tyr
  VARIANT 31: note = variant selected from the group consisting of Asn, Cys, Gln, Ser, Thr and Tyr
  VARIANT 39: note = variant selected from the group consisting of Asn, Cys, Gln, Ser, Thr and Tyr
  VARIANT 40: note = variant selected from the group consisting of Asn, Cys, Gln, Ser, Thr and Tyr
  VARIANT 41: note = variant selected from the group consisting of Asn, Cys, Gln, Ser, Thr and Tyr
  VARIANT 43: note = variant selected from the group consisting of Asn, Cys, Gln, Ser, Thr and Tyr
  VARIANT 44: note = variant selected from the group consisting of Asn, Cys, Gln, Ser, Thr and Tyr
  VARIANT 46: note = variant selected from the group consisting of Asn, Cys, Gln, Ser, Thr and Tyr
  VARIANT 51: note = variant selected from the group consisting of Asn, Cys, Gln, Ser, Thr and Tyr
  VARIANT 53: note = variant selected from the group consisting of Asn, Cys, Gln, Ser, Thr and Tyr
  VARIANT 54: note = variant selected from the group consisting of Asn, Cys, Gln, Ser, Thr and Tyr
  VARIANT 59: note = variant selected from the group consisting of Asn, Cys, Gln, Ser, Thr and Tyr
  VARIANT 60: note = variant selected from the group consisting of Asn, Cys, Gln, Ser, Thr and Tyr
  VARIANT 65: note = variant selected from the group consisting of Asn, Cys, Gln, Ser, Thr and Tyr
  VARIANT 66: note = variant selected from the group consisting of Asn, Cys, Gln, Ser, Thr and Tyr
  VARIANT 71: note = variant selected from the group consisting of Asn, Cys, Gln, Ser, Thr and Tyr
PXXPXXXPXXPXXPXXPXPXXXXXXPXXXXXXPXXPXPXXXPXXPXPXXPXPXXPXXPXXPXXPXXPXXPXPPXPPXXXXXXXXPXXPXXXX

SEQ ID NO: 2 - protein, 25 aa, synthetic construct
  VARIANT 2: note = variant selected from the group consisting of Ala, Ile, Leu, Met, Phe, Trp and Val
  VARIANT 3: note = variant selected from the group consisting of Ala, Ile, Leu, Met, Phe, Trp and Val
  VARIANT 8: note = variant selected from the group consisting of Ala, Ile, Leu, Met, Phe, Trp and Val
  VARIANT 9: note = variant selected from the group consisting of Ala, Ile, Leu, Met, Phe, Trp and Val
  VARIANT 14: note = variant selected from the group consisting of Ala, Ile, Leu, Met, Phe, Trp and Val
  VARIANT 15: note = variant selected from the group consisting of Ala, Ile, Leu, Met, Phe, Trp and Val
  VARIANT 23: note = variant selected from the group consisting of Ala, Ile, Leu, Met, Phe, Trp and Val
  VARIANT 5: note = variant selected from the group consisting of Asn, Cys, Gln, Ser, Thr and Tyr
  VARIANT 6: note = variant selected from the group consisting of Asn, Cys, Gln, Ser, Thr and Tyr
  VARIANT 11: note = variant selected from the group consisting of Asn, Cys, Gln, Ser, Thr and Tyr
  VARIANT 12: note = variant selected from the group consisting of Asn, Cys, Gln, Ser, Thr and Tyr
  VARIANT 17: note = variant selected from the group consisting of Asn, Cys, Gln, Ser, Thr and Tyr
  VARIANT 18: note = variant selected from the group consisting of Asn, Cys, Gln, Ser, Thr and Tyr
  VARIANT 20: note = variant selected from the group consisting of Asn, Cys, Gln, Ser, Thr and Tyr
PXXPXXPXXPXXPXXPXXPXPPXPP

SEQ ID NO: 3 - protein, 25 aa, synthetic construct
PLVPSYPLVPSYPLVPSYPYPPLPP

SEQ ID NO: 4 - protein, 25 aa, synthetic construct
PLVPSQPLVPSQPLVPSQPQPPLPP

SEQ ID NO: 5 - protein, 25 aa, synthetic construct
PHQPMQPQPPVHPMQPLPPQPPLPP

SEQ ID NO: 6 - protein, 25 aa, synthetic construct
PLVPSSPLVPSSPLVPSSPSPPLPP

SEQ ID NO: 7 - protein, 25 aa, synthetic construct
PLVPSSPLVPCCPLVPCCPSPPLPP